European Patent Application EP 4 467 570 A1, published November 27, 2024. Title: FUSION PROTEIN, AND PREPARATION METHOD THEREFOR AND USE THEREOF. Applicant: ZHU Daocheng. The sequence listing filed with the application follows.

SEQUENCE LISTING (4 sequences)

SEQ ID NO: 1 - protein, 554 aa, synthetic construct
  REGION 1..554: note = FP4
FTPPTVKILQSSCDGGGHFPPTIQLLCLVSGYTPGTINITWLEDGQVMDVDLSTASTTQEGELASTQSELTLSQKHWLSDRTYTCQVTYQGHTFEDSTKKCADSNPRGVSAYLSRPSPFDLFIRKSPTITCLVVDLAPSKGTVNLTWSRASGKPVNHSTRKEEKQRNGTLTVTSTLPVGTRDWIEGETYQCRVTHPHLPRALMRSTTKTSGPRAAPEVYAFATPEWPGSRDKRTLACLIQNFMPEDISVQWLHNEVQLPDARHSTTQPRKTKGSGFFVFSRLEVTRAEWEQKDEFICRAVHEAASPSQTVQRAVSVNPGKGSEPKSCDKTHTCPPCPAPELLGGPSVFLFPPKPKDTLMISRTPEVTCVVVDVSHEDPEVKFNWYVDGVEVHNAKTKPREEQYNSTYRVVSVLTVLHQDWLNGKEYKCKVSNKALPAPIEKTISKAKGQPREPQVYTLPPSRDELTKNQVSLTCLVKGFYPSDIAVEWESNGQPENNYKTTPPVLDSDGSFFLYSKLTVDKSRWQQGNVFSCSVMHEALHNHYTQKSLSLSPGK

SEQ ID NO: 2 - DNA, 1665 bp, synthetic construct
  misc_feature 1..1665: note = FP4
  source 1..1665: mol_type = other DNA
ttcaccccgcccaccgtgaagatcttacagtcgtcctgcgacggcggcgggcacttccccccgaccatccagctcctgtgcctcgtctctgggtacaccccagggactatcaacatcacctggctggaggacgggcaggtcatggacgtggacttgtccaccgcctctaccacgcaggagggtgagctggcctccacacaaagcgagctcaccctcagccagaagcactggctgtcagaccgcacctacacctgccaggtcacctatcaaggtcacacctttgaggacagcaccaagaagtgtgcagattccaacccgagaggggtgagcgcctacctaagccggcccagcccgttcgacctgttcatccgcaagtcgcccacgatcacctgtctggtggtggacctggcacccagcaaggggaccgtgaacctgacctggtcccgggccagtgggaagcctgtgaaccactccaccagaaaggaggagaagcagcgcaatggcacgttaaccgtcacgtccaccctgccggtgggcacccgagactggatcgagggggagacctaccagtgcagggtgacccacccccacctgcccagggccctcatgcggtccacgaccaagaccagcggcccgcgtgctgccccggaagtctatgcgtttgcgacgccggagtggccggggagccgggacaagcgcaccctcgcctgcctgatccagaacttcatgcctgaggacatctcggtgcagtggctgcacaacgaggtgcagctcccggacgcccggcacagcacgacgcagccccgcaagaccaagggctccggcttcttcgtcttcagccgtctagaggtgaccagggccgaatgggagcagaaagatgagttcatctgccgtgcagtccatgaggcagctagcccctcacagaccgtccagcgagcggtgtctgtaaatcccggtaaaggatccgagcccaaatcttgtgacaaaactcacacatgcccaccgtgcccagcacctgaactcctggggggaccgtcagtcttcctcttccccccaaaacccaaggacaccctcatgatctcccggacccctgaggtcacatgcgtggtggtggacgtgagccacgaagaccctgaggtcaagttcaactggtacgtggacggcgtggaggtgcataatgccaagacaaagccgcgggaggagcagtacaacagcacgtaccgggtggtcagcgtcctcaccgtcctgcaccaggactggctgaatggcaaggagtacaagtgcaaggtctccaacaaagccctcccagcccccatcgagaaaaccatctccaaagccaaagggcagccccgagaaccacaggtgtacaccctgcccccatcccgggatgagctgaccaagaaccaggtcagcctgacctgcctggtcaaaggcttctatcccagcgacatcgccgtggagtgggagagcaatgggcagccggagaacaactacaagaccacgcctcccgtgctggactccgacggctccttcttcctctacagcaagctcaccgtggacaagagcaggtggcagcaggggaacgtcttctcatgctccgtgatgcatgaggctctgcacaaccactacacgcagaagagcctctccctgtctccgggtaaatga

SEQ ID NO: 3 - protein, 552 aa, synthetic construct
  REGION 1..552: note = MEG
FTPPTVKILQSSCDGGGHFPPTIQLLCLVSGYTPGTINITWLEDGQVMDVDLSTASTTQEGELASTQSELTLSQKHWLSDRTYTCQVTYQGHTFEDSTKKCADSNPRGVSAYLSRPSPFDLFIRKSPTITCLVVDLAPSKGTVNLTWSRASGKPVNHSTRKEEKQRNGTLTVTSTLPVGTRDWIEGETYQCRVTHPHLPRALMRSTTKTSGPRAAPEVYAFATPEWPGSRDKRTLACLIQNFMPEDISVQWLHNEVQLPDARHSTTQPRKTKGSGFFVFSRLEVTRAEWEQKDEFICRAVHEAASPSQTVQRAVSVNPGKEPKSCDKTHTCPPCPAPELLGGDSVFLFPPKPKDTLMISRTPEVTCVVVDVSHEDPEVKFNWYVDGVEVHNAKTKPREEQYNSTYRVVSVLTVLHQDWLNGKEYKCKVSNKALPAPIEKTISKAKGQPREPQVYTLPPSRDELTKNQVSLTCLVKGFYPSDIAVEWESNGQPENNYKTTPPVLDSDGSFFLYSKLTVDKSRWQQGNVFSCSVMHEALHNHYTQKSLSLSPGK

SEQ ID NO: 4 - DNA, 1659 bp, synthetic construct
  misc_feature 1..1659: note = MEG
  source 1..1659: mol_type = other DNA
ttcaccccgcccaccgtgaagatcttacagtcgtcctgcgacggcggcgggcacttccccccgaccatccagctcctgtgcctcgtctctgggtacaccccagggactatcaacatcacctggctggaggacgggcaggtcatggacgtggacttgtccaccgcctctaccacgcaggagggtgagctggcctccacacaaagcgagctcaccctcagccagaagcactggctgtcagaccgcacctacacctgccaggtcacctatcaaggtcacacctttgaggacagcaccaagaagtgtgcagattccaacccgagaggggtgagcgcctacctaagccggcccagcccgttcgacctgttcatccgcaagtcgcccacgatcacctgtctggtggtggacctggcacccagcaaggggaccgtgaacctgacctggtcccgggccagtgggaagcctgtgaaccactccaccagaaaggaggagaagcagcgcaatggcacgttaaccgtcacgtccaccctgccggtgggcacccgagactggatcgagggggagacctaccagtgcagggtgacccacccccacctgcccagggccctcatgcggtccacgaccaagaccagcggcccgcgtgctgccccggaagtctatgcgtttgcgacgccggagtggccggggagccgggacaagcgcaccctcgcctgcctgatccagaacttcatgcctgaggacatctcggtgcagtggctgcacaacgaggtgcagctcccggacgcccggcacagcacgacgcagccccgcaagaccaagggctccggcttcttcgtcttcagccgcctggaggtgaccagggccgaatgggagcagaaagatgagttcatctgccgtgcagtccatgaggcagctagcccctcacagaccgtccagcgagcggtgtctgtaaatcccggtaaagagcccaaatcttgtgacaaaactcacacatgcccaccgtgcccagcacctgaactcctggggggagactcagtcttcctcttccccccaaaacccaaggacaccctcatgatctcccggacccctgaggtcacatgcgtggtggtggacgtgagccacgaagaccctgaggtcaagttcaactggtacgtggacggcgtggaggtgcataatgccaagacaaagccgcgggaggagcagtacaacagcacgtaccgtgtggtcagcgtcctcaccgtcctgcaccaggactggctgaatggcaaggagtacaagtgcaaggtctccaacaaagccctcccagcccccatcgagaaaaccatctccaaagccaaagggcagccccgagaaccacaggtgtacaccctgcccccatcccgggatgagctgaccaagaaccaggtcagcctgacctgcctggtcaaaggcttctatcccagcgacatcgccgtggagtgggagagcaatgggcagccggagaacaactacaagaccacgcctcccgtgctggactccgacggctccttcttcctctacagcaagctcaccgtggacaagagcaggtggcagcaggggaacgtcttctcatgctccgtgatgcatgaggctctgcacaaccactacacgcagaagagcctctccctgtctccgggtaaatga